European Patent Specification EP 3 628 321 B1, published September 6, 2023. Title: COMPOUNDS AND METHODS FOR ENHANCING ERYTHROPOIESIS. Applicant: Wu, Rong-Tsun. The sequence listing filed with the application follows.

SEQUENCE LISTING (8 sequences)

SEQ ID NO: 1 - DNA, 20 bp, Artificial Sequence
  primer
gtgggccgccctaggcacca

SEQ ID NO: 2 - DNA, 20 bp, Artificial Sequence
  primer
tggccttagggttcaggggg

SEQ ID NO: 3 - DNA, 20 bp, Artificial Sequence
  primer
aatggaggtggaagaacagg

SEQ ID NO: 4 - DNA, 19 bp, Artificial Sequence
  primer
acccgaagcagtgaagtga

SEQ ID NO: 5 - DNA, 20 bp, Artificial Sequence
  primer
tggcatcgtggaagggctca

SEQ ID NO: 6 - DNA, 20 bp, Artificial Sequence
  primer
ggaagaatgggagttgctgt

SEQ ID NO: 7 - DNA, 21 bp, Artificial Sequence
  primer
cttggcatccacgatgttcat

SEQ ID NO: 8 - DNA, 21 bp, Artificial Sequence
  primer
tggtgctgactgcatttctca